European Patent Specification EP 3 673 086 B1, published April 9, 2025. Title: ELECTROCHEMICAL DETECTION OF BACTERIAL AND/OR FUNGAL INFECTIONS. Applicant: Clinical Micro Systems, Inc. (dba GenMark Diagnostics, Inc.) Freeman-Cook, Lisa L Shaw, Christine J Martinez, Milena I Al-Khouri, Anna M Brown, Bradley A. Harvey, John J. The sequence listing filed with the application follows.

SEQUENCE LISTING (9 sequences)

SEQ ID NO: 1 - DNA, 25 bp, Rhodotorula
  misc_feature (1)..(1): n is a, c, g, or t
nactagcactacacgagcacggaag

SEQ ID NO: 2 - DNA, 25 bp, rhodotorula
  misc_feature (1)..(1): n is a, c, g, or t
nagcacggaagtagtaacccattag

SEQ ID NO: 3 - DNA, 26 bp, trichosporon
actctacaccgattcttctaacttca

SEQ ID NO: 4 - DNA, 26 bp, trichosporon
acacttcaccgattcttctaacttca

SEQ ID NO: 5 - DNA, 24 bp, rhodotorula
ggtagttcggagcgtggaatacca

SEQ ID NO: 6 - DNA, 24 bp, rhodotorula
ggtcgtttggtacgtagaatacca

SEQ ID NO: 7 - DNA, 27 bp, trichosporon
  misc_feature (1)..(1): n is a, c, g, or t
natgtaatatggatgcattggaactcg

SEQ ID NO: 8 - DNA, 27 bp, trichosporon
  misc_feature (1)..(1): n is a, c, g, or t
natgtaatatggatgcattggcactcg

SEQ ID NO: 9 - DNA, 27 bp, trichosporon
  misc_feature (1)..(1): n is a, c, g, or t
natataataaggatgcattggaattcg